European Patent Application EP 4 681 740 A1, published January 21, 2026. Title: COMBINATION OF ANTI-CDH6 ANTIBODY-DRUG CONJUGATE WITH VEGF INHIBITOR. Applicant: DAIICHI SANKYO COMPANY, LIMITED. Application EP 24770920.7, filed March 13, 2024. The sequence listing filed with the application follows.

SEQUENCE LISTING (41 sequences)

SEQ ID NO: 1 - protein, 115 aa, Homo sapiens
  REGION 1..115: note = Human CDH6 EC3
PQSTYQFKTPESSPPGTPIGRIKASDADVGENAEIEYSITDGEGLDMFDVITDQETQEGIITVKKLLDFEKKKVYTLKVEASNPYVEPRFLYLGPFKDSATVRIVVEDVDEPPVF

SEQ ID NO: 2 - protein, 10 aa, Rattus norvegicus
  REGION 1..10: note = amino acid sequence of chG019 CDRH1
GYTFTRNFMH

SEQ ID NO: 3 - protein, 10 aa, synthetic construct
  REGION 1..10: note = amino acid sequence of chG019 CDRH2
WIYPGDGETE

SEQ ID NO: 4 - protein, 13 aa, Rattus norvegicus
  REGION 1..13: note = amino acid sequence of chG019 CDRH3
GVYGGFAGGYFDF

SEQ ID NO: 5 - protein, 11 aa, Rattus norvegicus
  REGION 1..11: note = amino acid sequence of chG019 CDRL1
KASQNIYKNLA

SEQ ID NO: 6 - protein, 7 aa, Rattus norvegicus
  REGION 1..7: note = amino acid sequence of chG019 CDRL2
DANTLQT

SEQ ID NO: 7 - protein, 8 aa, Rattus norvegicus
  REGION 1..8: note = amino acid sequence of chG019 CDRL3
QQYYSGWA

SEQ ID NO: 8 - protein, 10 aa, Rattus norvegicus
  REGION 1..10: note = amino acid sequence of rG019 CDRH2
WIYCGDGETE

SEQ ID NO: 9 - protein, 10 aa, Rattus norvegicus
  REGION 1..10: note = amino acid sequence of rG055 CDRH1
DYSITSNYWG

SEQ ID NO: 10 - protein, 9 aa, Rattus norvegicus
  REGION 1..9: note = amino acid sequence of rG055 CDRH2
YITYSGYTS

SEQ ID NO: 11 - protein, 13 aa, Rattus norvegicus
  REGION 1..13: note = amino acid sequence of rG055 CDRH3
SINHGGYSYVVDA

SEQ ID NO: 12 - protein, 11 aa, Rattus norvegicus
  REGION 1..11: note = amino acid sequence of rG055 CDRL1
KTSKNISNYLV

SEQ ID NO: 13 - protein, 7 aa, Rattus norvegicus
  REGION 1..7: note = amino acid sequence of rG055 CDRL2
SGSTLQS

SEQ ID NO: 14 - protein, 9 aa, Rattus norvegicus
  REGION 1..9: note = amino acid sequence of rG055 CDRL3
QQYYEKPFT

SEQ ID NO: 15 - protein, 10 aa, Rattus norvegicus
  REGION 1..10: note = amino acid sequence of rG056 CDRH1
DYSITTYFWG

SEQ ID NO: 16 - protein, 9 aa, Rattus norvegicus
  REGION 1..9: note = amino acid sequence of rG056 CDRH2
YMSYRGGTS

SEQ ID NO: 17 - protein, 13 aa, Rattus norvegicus
  REGION 1..13: note = amino acid sequence of rG056 CDRH3
CPNYGGHSLVFDY

SEQ ID NO: 18 - protein, 11 aa, Rattus norvegicus
  REGION 1..11: note = amino acid sequence of rG056 CDRL1
RATKSIGIYLA

SEQ ID NO: 19 - protein, 7 aa, Rattus norvegicus
  REGION 1..7: note = amino acid sequence of rG056 CDRL2
SGSTLQS

SEQ ID NO: 20 - protein, 9 aa, Rattus norvegicus
  REGION 1..9: note = amino acid sequence of rG056 CDRL3
QQFYENPFT

SEQ ID NO: 21 - protein, 10 aa, Rattus norvegicus
  REGION 1..10: note = amino acid sequence of rG061 CDRH1
GYSITTYYWG

SEQ ID NO: 22 - protein, 9 aa, Rattus norvegicus
  REGION 1..9: note = amino acid sequence of rG061 CDRH2
YISYSGRTS

SEQ ID NO: 23 - protein, 13 aa, Rattus norvegicus
  REGION 1..13: note = amino acid sequence of rG061 CDRH3
SPINHGGYWYFDF

SEQ ID NO: 24 - protein, 11 aa, Rattus norvegicus
  REGION 1..11: note = amino acid sequence of rG061 CDRL1
KATKSISNYLA

SEQ ID NO: 25 - protein, 7 aa, Rattus norvegicus
  REGION 1..7: note = amino acid sequence of rG061 CDRL2
SGSTLQS

SEQ ID NO: 26 - protein, 9 aa, Rattus norvegicus
  REGION 1..9: note = amino acid sequence of rG061 CDRL3
QQYYEKPLT

SEQ ID NO: 27 - protein, 471 aa, synthetic construct
  REGION 1..471: note = amino acid sequence of hH01 heavy chain full-length
MKHLWFFLLLVAAPRWVLSEVQLVQSGAEVKKPGASVKVSCKASGYTFTRNFMHWVRQAPGQGLEWMGWIYPGDGETEYAQKFQGRVTITADTSTSTAYMELSSLRSEDTAVYYCARGVYGGFAGGYFDFWGQGTLVTVSSASTKGPSVFPLAPSSKSTSGGTAALGCLVKDYFPEPVTVSWNSGALTSGVHTFPAVLQSSGLYSLSSVVTVPSSSLGTQTYICNVNHKPSNTKVDKRVEPKSCDKTHTCPPCPAPELLGGPSVFLFPPKPKDTLMISRTPEVTCVVVDVSHEDPEVKFNWYVDGVEVHNAKTKPREEQYNSTYRVVSVLTVLHQDWLNGKEYKCKVSNKALPAPIEKTISKAKGQPREPQVYTLPPSREEMTKNQVSLTCLVKGFYPSDIAVEWESNGQPENNYKTTPPVLDSDGSFFLYSKLTVDKSRWQQGNVFSCSVMHEALHNHYTQKSLSLSPGK

SEQ ID NO: 28 - protein, 122 aa, synthetic construct
  REGION 1..122: note = amino acid sequence of hH01 heavy chain variable region
EVQLVQSGAEVKKPGASVKVSCKASGYTFTRNFMHWVRQAPGQGLEWMGWIYPGDGETEYAQKFQGRVTITADTSTSTAYMELSSLRSEDTAVYYCARGVYGGFAGGYFDFWGQGTLVTVSS

SEQ ID NO: 29 - protein, 452 aa, synthetic construct
  REGION 1..452: note = Matured heavy chain amino acid sequence of hH01 heavy chain, without a signal sequence
EVQLVQSGAEVKKPGASVKVSCKASGYTFTRNFMHWVRQAPGQGLEWMGWIYPGDGETEYAQKFQGRVTITADTSTSTAYMELSSLRSEDTAVYYCARGVYGGFAGGYFDFWGQGTLVTVSSASTKGPSVFPLAPSSKSTSGGTAALGCLVKDYFPEPVTVSWNSGALTSGVHTFPAVLQSSGLYSLSSVVTVPSSSLGTQTYICNVNHKPSNTKVDKRVEPKSCDKTHTCPPCPAPELLGGPSVFLFPPKPKDTLMISRTPEVTCVVVDVSHEDPEVKFNWYVDGVEVHNAKTKPREEQYNSTYRVVSVLTVLHQDWLNGKEYKCKVSNKALPAPIEKTISKAKGQPREPQVYTLPPSREEMTKNQVSLTCLVKGFYPSDIAVEWESNGQPENNYKTTPPVLDSDGSFFLYSKLTVDKSRWQQGNVFSCSVMHEALHNHYTQKSLSLSPGK

SEQ ID NO: 30 - protein, 471 aa, synthetic construct
  REGION 1..471: note = amino acid sequence of hH02 heavy chain full-length
MKHLWFFLLLVAAPRWVLSEVQLVQSGAEVKKPGASVKVSCKASGYTFTRNFMHWVRQAPGQGLEWMGWIYPGDGETEYNQKFQGRVTITADRSTSTAYMELSSLRSEDTAVYFCARGVYGGFAGGYFDFWGQGTLVTVSSASTKGPSVFPLAPSSKSTSGGTAALGCLVKDYFPEPVTVSWNSGALTSGVHTFPAVLQSSGLYSLSSVVTVPSSSLGTQTYICNVNHKPSNTKVDKRVEPKSCDKTHTCPPCPAPELLGGPSVFLFPPKPKDTLMISRTPEVTCVVVDVSHEDPEVKFNWYVDGVEVHNAKTKPREEQYNSTYRVVSVLTVLHQDWLNGKEYKCKVSNKALPAPIEKTISKAKGQPREPQVYTLPPSREEMTKNQVSLTCLVKGFYPSDIAVEWESNGQPENNYKTTPPVLDSDGSFFLYSKLTVDKSRWQQGNVFSCSVMHEALHNHYTQKSLSLSPGK

SEQ ID NO: 31 - protein, 122 aa, synthetic construct
  REGION 1..122: note = amino acid sequence of hH02 heavy chain variable region
EVQLVQSGAEVKKPGASVKVSCKASGYTFTRNFMHWVRQAPGQGLEWMGWIYPGDGETEYNQKFQGRVTITADRSTSTAYMELSSLRSEDTAVYFCARGVYGGFAGGYFDFWGQGTLVTVSS

SEQ ID NO: 32 - protein, 452 aa, synthetic construct
  REGION 1..451: note = Matured heavy chain amino acid sequence of hH02 heavy chain, without a signal sequence
EVQLVQSGAEVKKPGASVKVSCKASGYTFTRNFMHWVRQAPGQGLEWMGWIYPGDGETEYNQKFQGRVTITADRSTSTAYMELSSLRSEDTAVYFCARGVYGGFAGGYFDFWGQGTLVTVSSASTKGPSVFPLAPSSKSTSGGTAALGCLVKDYFPEPVTVSWNSGALTSGVHTFPAVLQSSGLYSLSSVVTVPSSSLGTQTYICNVNHKPSNTKVDKRVEPKSCDKTHTCPPCPAPELLGGPSVFLFPPKPKDTLMISRTPEVTCVVVDVSHEDPEVKFNWYVDGVEVHNAKTKPREEQYNSTYRVVSVLTVLHQDWLNGKEYKCKVSNKALPAPIEKTISKAKGQPREPQVYTLPPSREEMTKNQVSLTCLVKGFYPSDIAVEWESNGQPENNYKTTPPVLDSDGSFFLYSKLTVDKSRWQQGNVFSCSVMHEALHNHYTQKSLSLSPGK

SEQ ID NO: 33 - protein, 471 aa, synthetic construct
  REGION 1..471: note = amino acid sequence of hH04 heavy chain full-length
MKHLWFFLLLVAAPRWVLSQVQLVQSGAEVKKPGASVKVSCKASGYTFTRNFMHWIRQAPGQGLEWMGWIYPGDGETEYAQKFQGRVTLTADRSTSTAYMELSSLRSEDTAVYYCARGVYGGFAGGYFDFWGQGTLVTVSSASTKGPSVFPLAPSSKSTSGGTAALGCLVKDYFPEPVTVSWNSGALTSGVHTFPAVLQSSGLYSLSSVVTVPSSSLGTQTYICNVNHKPSNTKVDKRVEPKSCDKTHTCPPCPAPELLGGPSVFLFPPKPKDTLMISRTPEVTCVVVDVSHEDPEVKFNWYVDGVEVHNAKTKPREEQYNSTYRVVSVLTVLHQDWLNGKEYKCKVSNKALPAPIEKTISKAKGQPREPQVYTLPPSREEMTKNQVSLTCLVKGFYPSDIAVEWESNGQPENNYKTTPPVLDSDGSFFLYSKLTVDKSRWQQGNVFSCSVMHEALHNHYTQKSLSLSPGK

SEQ ID NO: 34 - protein, 122 aa, synthetic construct
  REGION 1..122: note = amino acid sequence of hH04 heavy chain variable region
QVQLVQSGAEVKKPGASVKVSCKASGYTFTRNFMHWIRQAPGQGLEWMGWIYPGDGETEYAQKFQGRVTLTADRSTSTAYMELSSLRSEDTAVYYCARGVYGGFAGGYFDFWGQGTLVTVSS

SEQ ID NO: 35 - protein, 452 aa, synthetic construct
  REGION 1..452: note = Matured heavy chain amino acid sequence of hH04 heavy chain, without a signal sequence
QVQLVQSGAEVKKPGASVKVSCKASGYTFTRNFMHWIRQAPGQGLEWMGWIYPGDGETEYAQKFQGRVTLTADRSTSTAYMELSSLRSEDTAVYYCARGVYGGFAGGYFDFWGQGTLVTVSSASTKGPSVFPLAPSSKSTSGGTAALGCLVKDYFPEPVTVSWNSGALTSGVHTFPAVLQSSGLYSLSSVVTVPSSSLGTQTYICNVNHKPSNTKVDKRVEPKSCDKTHTCPPCPAPELLGGPSVFLFPPKPKDTLMISRTPEVTCVVVDVSHEDPEVKFNWYVDGVEVHNAKTKPREEQYNSTYRVVSVLTVLHQDWLNGKEYKCKVSNKALPAPIEKTISKAKGQPREPQVYTLPPSREEMTKNQVSLTCLVKGFYPSDIAVEWESNGQPENNYKTTPPVLDSDGSFFLYSKLTVDKSRWQQGNVFSCSVMHEALHNHYTQKSLSLSPGK

SEQ ID NO: 36 - protein, 233 aa, synthetic construct
  REGION 1..233: note = amino acid sequence of hL02 light chain full-length
MVLQTQVFISLLLWISGAYGDIQMTQSPSSLSASVGDRVTITCKASQNIYKNLAWYQQKPGKAPKLLIYDANTLQTGVPSRFSGSGSGSDFTLTISSLQPEDFATYFCQQYYSGWAFGQGTKVEIKRTVAAPSVFIFPPSDEQLKSGTASVVCLLNNFYPREAKVQWKVDNALQSGNSQESVTEQDSKDSTYSLSSTLTLSKADYEKHKVYACEVTHQGLSSPVTKSFNRGEC

SEQ ID NO: 37 - protein, 108 aa, synthetic construct
  REGION 1..108: note = amino acid sequence of hL02 light chain variable region
DIQMTQSPSSLSASVGDRVTITCKASQNIYKNLAWYQQKPGKAPKLLIYDANTLQTGVPSRFSGSGSGSDFTLTISSLQPEDFATYFCQQYYSGWAFGQGTKVEIKRT

SEQ ID NO: 38 - protein, 213 aa, synthetic construct
  REGION 1..213: note = Matured light chain amino acid sequence of hL02 light chain, without a signal sequence
DIQMTQSPSSLSASVGDRVTITCKASQNIYKNLAWYQQKPGKAPKLLIYDANTLQTGVPSRFSGSGSGSDFTLTISSLQPEDFATYFCQQYYSGWAFGQGTKVEIKRTVAAPSVFIFPPSDEQLKSGTASVVCLLNNFYPREAKVQWKVDNALQSGNSQESVTEQDSKDSTYSLSSTLTLSKADYEKHKVYACEVTHQGLSSPVTKSFNRGEC

SEQ ID NO: 39 - protein, 233 aa, synthetic construct
  REGION 1..233: note = amino acid sequence of hL03 light chain full-length
MVLQTQVFISLLLWISGAYGDIQMTQSPSSLSASVGDRVTITCKASQNIYKNLAWYQQKLGEGPKLLIYDANTLQTGVPSRFSGSGSGTDFTLTISSLQPEDFATYYCQQYYSGWAFGQGTKVEIKRTVAAPSVFIFPPSDEQLKSGTASVVCLLNNFYPREAKVQWKVDNALQSGNSQESVTEQDSKDSTYSLSSTLTLSKADYEKHKVYACEVTHQGLSSPVTKSFNRGEC

SEQ ID NO: 40 - protein, 108 aa, synthetic construct
  REGION 1..108: note = amino acid sequence of hL03 light chain variable region
DIQMTQSPSSLSASVGDRVTITCKASQNIYKNLAWYQQKLGEGPKLLIYDANTLQTGVPSRFSGSGSGTDFTLTISSLQPEDFATYYCQQYYSGWAFGQGTKVEIKRT

SEQ ID NO: 41 - protein, 213 aa, synthetic construct
  REGION 1..213: note = Matured light chain amino acid sequence of hL03 light chain, without a signal sequence
DIQMTQSPSSLSASVGDRVTITCKASQNIYKNLAWYQQKLGEGPKLLIYDANTLQTGVPSRFSGSGSGTDFTLTISSLQPEDFATYYCQQYYSGWAFGQGTKVEIKRTVAAPSVFIFPPSDEQLKSGTASVVCLLNNFYPREAKVQWKVDNALQSGNSQESVTEQDSKDSTYSLSSTLTLSKADYEKHKVYACEVTHQGLSSPVTKSFNRGEC